European Patent Application EP 4 650 361 A1, published November 19, 2025. Title: ARGININE OPTICAL PROBE. Applicant: EAST CHINA UNIVERSITY OF SCIENCE AND TECHNOLOGY. The sequence listing filed with the application follows.

SEQUENCE LISTING (15 sequences)

SEQ ID NO: 1 - protein, 229 aa, synthetic construct
ASVSARTLHFGTSATYAPYEFVDADNKIVGFDIDVANAVCKEMQAECSFTNQSFDSLIPSLRFKKFDAVIAGMDMTPKREQQVSFSQPYYEGLSAVVVTRKGAYHTFADLKGKKVGLENGTTHQRYLQDKQQAITPVAYDSYLNAFTDLKNNRLEGVFGDVAAIGKWLKNNPDYAIMDERASDPDYYGKGLGIAVRKDNDALLQEINAALDKVKASPEYAQMQEKWFTQ

SEQ ID NO: 2 - protein, 473 aa, synthetic construct
ASVSARTLHFGTSATYAPYEFVDADNKIVGFDIDVANAVCKEMQAECSFTNQSFDSLIPSLRFKKFDAVIAGMDMTPKREQQVSFSQPYYEGLSAVVVTRKGAYHTFADLKGKKVGLENGTTHQRYLQDKQQAITPVAYDSYLNAFTDLKNNRLEGVFGDVAAIGKWLKNNPDYAIMDERASDYNSDNVYIMADKQKNGIKANFKIRHNVEDGSVQLADHYQQNTPIGDGPVLLPDNHYLSFQSVLSKDPNEKRDHMVLLEFVTAAGITLGMDELYNVDGGSGGTGSKGEELFTGVVPILVELDGDVNGHKFSVSGEGEGDATYGKLTLKLICTTGKLPVPWPTLVTTLGYGLKCFARYPDHMKQHDFFKSAMPEGYVQERTIFFKDDGNYKTRAEVKFEGDTLVNRIELKGIGFKEDGNILGHKLEYNYYGKGLGIAVRKDNDALLQEINAALDKVKASPEYAQMQEKWFTQ

SEQ ID NO: 3 - protein, 246 aa, synthetic construct
YNSDNVYIMADKQKNGIKANFKIRHNVEDGSVQLADHYQQNTPIGDGPVLLPDNHYLSFQSVLSKDPNEKRDHMVLLEFVTAAGITLGMDELYNVDGGSGGTGSKGEELFTGVVPILVELDGDVNGHKFSVSGEGEGDATYGKLTLKLICTTGKLPVPWPTLVTTLGYGLKCFARYPDHMKQHDFFKSAMPEGYVQERTIFFKDDGNYKTRAEVKFEGDTLVNRIELKGIDFKEDGNILGHKLEYN

SEQ ID NO: 4 - protein, 473 aa, synthetic construct
ASVSARTLHFGTSAAYAPYEFVDADNKIVGFDIDVANAVCKEMQAECSFTNQSFDSLIPSLRFKKFDAVIAGMDMTPKREQQVSFSQPYYEGLSAVVVTRKGAYHTFADLKGKKVGLENGTTHQRYLQDKQQAITPVAYDSYLNAFTDLKNNRLEGVFGDVAAIGKWLKNNPDYAIMDERASDYNSDNVYIMADKQKNGIKANFKIRHNVEDGSVQLADHYQQNTPIGDGPVLLPDNHYLSFQSVLSKDPNEKRDHMVLLEFVTAAGITLGMDELYNVDGGSGGTGSKGEELFTGVVPILVELDGDVNGHKFSVSGEGEGDATYGKLTLKLICTTGKLPVPWPTLVTTLGYGLKCFARYPDHMKQHDFFKSAMPEGYVQERTIFFKDDGNYKTRAEVKFEGDTLVNRIELKGIGFKEDGNILGHKLEYNYYGKGLGIAVRKDNDALLQEINAALDKVKASPEYAQMQEKWFTQ

SEQ ID NO: 5 - protein, 473 aa, synthetic construct
ASVSARTLHFGTSATYAPYAFVDADNKIVGFDIDVANAVCKEMQAECSFTNQSFDSLIPSLRFKKFDAVIAGMDMTPKREQQVSFSQPYYEGLSAVVVTRKGAYHTFADLKGKKVGLENGTTHQRYLQDKQQAITPVAYDSYLNAFTDLKNNRLEGVFGDVAAIGKWLKNNPDYAIMDERASDYNSDNVYIMADKQKNGIKANFKIRHNVEDGSVQLADHYQQNTPIGDGPVLLPDNHYLSFQSVLSKDPNEKRDHMVLLEFVTAAGITLGMDELYNVDGGSGGTGSKGEELFTGVVPILVELDGDVNGHKFSVSGEGEGDATYGKLTLKLICTTGKLPVPWPTLVTTLGYGLKCFARYPDHMKQHDFFKSAMPEGYVQERTIFFKDDGNYKTRAEVKFEGDTLVNRIELKGIGFKEDGNILGHKLEYNYYGKGLGIAVRKDNDALLQEINAALDKVKASPEYAQMQEKWFTQ

SEQ ID NO: 6 - protein, 473 aa, synthetic construct
ASVSARTLHFGTSATYAPYEFVDADNKIVGFDIDVANAVCKEMQAECSFTNQSADSLIPSLRFKKFDAVIAGMDMTPKREQQVSFSQPYYEGLSAVVVTRKGAYHTFADLKGKKVGLENGTTHQRYLQDKQQAITPVAYDSYLNAFTDLKNNRLEGVFGDVAAIGKWLKNNPDYAIMDERASDYNSDNVYIMADKQKNGIKANFKIRHNVEDGSVQLADHYQQNTPIGDGPVLLPDNHYLSFQSVLSKDPNEKRDHMVLLEFVTAAGITLGMDELYNVDGGSGGTGSKGEELFTGVVPILVELDGDVNGHKFSVSGEGEGDATYGKLTLKLICTTGKLPVPWPTLVTTLGYGLKCFARYPDHMKQHDFFKSAMPEGYVQERTIFFKDDGNYKTRAEVKFEGDTLVNRIELKGIGFKEDGNILGHKLEYNYYGKGLGIAVRKDNDALLQEINAALDKVKASPEYAQMQEKWFTQ

SEQ ID NO: 7 - protein, 473 aa, synthetic construct
ASVSARTLHFGTSATYAPYEFVDADNKIVGFDIDVANAVCKEMQAECSFTNQSFDSLIPSLRFKKFDAVIAAMDMTPKREQQVSFSQPYYEGLSAVVVTRKGAYHTFADLKGKKVGLENGTTHQRYLQDKQQAITPVAYDSYLNAFTDLKNNRLEGVFGDVAAIGKWLKNNPDYAIMDERASDYNSDNVYIMADKQKNGIKANFKIRHNVEDGSVQLADHYQQNTPIGDGPVLLPDNHYLSFQSVLSKDPNEKRDHMVLLEFVTAAGITLGMDELYNVDGGSGGTGSKGEELFTGVVPILVELDGDVNGHKFSVSGEGEGDATYGKLTLKLICTTGKLPVPWPTLVTTLGYGLKCFARYPDHMKQHDFFKSAMPEGYVQERTIFFKDDGNYKTRAEVKFEGDTLVNRIELKGIGFKEDGNILGHKLEYNYYGKGLGIAVRKDNDALLQEINAALDKVKASPEYAQMQEKWFTQ

SEQ ID NO: 8 - protein, 473 aa, synthetic construct
ASVSARTLHFGTSATYAPYEFVDADNKIVGFDIDVANAVCKEMQAECSFTNQSFDSLIPSLRFKKFDAVIAGADMTPKREQQVSFSQPYYEGLSAVVVTRKGAYHTFADLKGKKVGLENGTTHQRYLQDKQQAITPVAYDSYLNAFTDLKNNRLEGVFGDVAAIGKWLKNNPDYAIMDERASDYNSDNVYIMADKQKNGIKANFKIRHNVEDGSVQLADHYQQNTPIGDGPVLLPDNHYLSFQSVLSKDPNEKRDHMVLLEFVTAAGITLGMDELYNVDGGSGGTGSKGEELFTGVVPILVELDGDVNGHKFSVSGEGEGDATYGKLTLKLICTTGKLPVPWPTLVTTLGYGLKCFARYPDHMKQHDFFKSAMPEGYVQERTIFFKDDGNYKTRAEVKFEGDTLVNRIELKGIGFKEDGNILGHKLEYNYYGKGLGIAVRKDNDALLQEINAALDKVKASPEYAQMQEKWFTQ

SEQ ID NO: 9 - protein, 473 aa, synthetic construct
ASVSARTLHFGTSATYAPYEFVDADNKIVGFDIDVANAVCKEMQAECSFTNQSFDSLIPSLRFKKFDAVIAGMAMTPKREQQVSFSQPYYEGLSAVVVTRKGAYHTFADLKGKKVGLENGTTHQRYLQDKQQAITPVAYDSYLNAFTDLKNNRLEGVFGDVAAIGKWLKNNPDYAIMDERASDYNSDNVYIMADKQKNGIKANFKIRHNVEDGSVQLADHYQQNTPIGDGPVLLPDNHYLSFQSVLSKDPNEKRDHMVLLEFVTAAGITLGMDELYNVDGGSGGTGSKGEELFTGVVPILVELDGDVNGHKFSVSGEGEGDATYGKLTLKLICTTGKLPVPWPTLVTTLGYGLKCFARYPDHMKQHDFFKSAMPEGYVQERTIFFKDDGNYKTRAEVKFEGDTLVNRIELKGIGFKEDGNILGHKLEYNYYGKGLGIAVRKDNDALLQEINAALDKVKASPEYAQMQEKWFTQ

SEQ ID NO: 10 - protein, 473 aa, synthetic construct
ASVSARTLHFGTSATYAPYEFVDADNKIVGFDIDVANAVCKEMQAECSFTNQSFDSLIPSLRFKKFDAVIAGMDMTPKAEQQVSFSQPYYEGLSAVVVTRKGAYHTFADLKGKKVGLENGTTHQRYLQDKQQAITPVAYDSYLNAFTDLKNNRLEGVFGDVAAIGKWLKNNPDYAIMDERASDYNSDNVYIMADKQKNGIKANFKIRHNVEDGSVQLADHYQQNTPIGDGPVLLPDNHYLSFQSVLSKDPNEKRDHMVLLEFVTAAGITLGMDELYNVDGGSGGTGSKGEELFTGVVPILVELDGDVNGHKFSVSGEGEGDATYGKLTLKLICTTGKLPVPWPTLVTTLGYGLKCFARYPDHMKQHDFFKSAMPEGYVQERTIFFKDDGNYKTRAEVKFEGDTLVNRIELKGIGFKEDGNILGHKLEYNYYGKGLGIAVRKDNDALLQEINAALDKVKASPEYAQMQEKWFTQ

SEQ ID NO: 11 - protein, 473 aa, synthetic construct
ASVSARTLHFGTSATYAPYEFVDADNKIVGFDIDVANAVCKEMQAECSFTNQSFDSLIPSLRFKKFDAVIAGMDMTPKREQQVSFSQPYYEGLSAVVVTRKGAYHTFADLKGKKVGLANGTTHQRYLQDKQQAITPVAYDSYLNAFTDLKNNRLEGVFGDVAAIGKWLKNNPDYAIMDERASDYNSDNVYIMADKQKNGIKANFKIRHNVEDGSVQLADHYQQNTPIGDGPVLLPDNHYLSFQSVLSKDPNEKRDHMVLLEFVTAAGITLGMDELYNVDGGSGGTGSKGEELFTGVVPILVELDGDVNGHKFSVSGEGEGDATYGKLTLKLICTTGKLPVPWPTLVTTLGYGLKCFARYPDHMKQHDFFKSAMPEGYVQERTIFFKDDGNYKTRAEVKFEGDTLVNRIELKGIGFKEDGNILGHKLEYNYYGKGLGIAVRKDNDALLQEINAALDKVKASPEYAQMQEKWFTQ

SEQ ID NO: 12 - protein, 473 aa, synthetic construct
ASVSARTLHFGTSATYAPYEFVDADNKIVGFDIDVANAVCKEMQAECSFTNQSFDSLIPSLRFKKFDAVIAGMDMTPKREQQVSFSQPYYEGLSAVVVTRKGAYHTFADLKGKKVGLENGATHQRYLQDKQQAITPVAYDSYLNAFTDLKNNRLEGVFGDVAAIGKWLKNNPDYAIMDERASDYNSDNVYIMADKQKNGIKANFKIRHNVEDGSVQLADHYQQNTPIGDGPVLLPDNHYLSFQSVLSKDPNEKRDHMVLLEFVTAAGITLGMDELYNVDGGSGGTGSKGEELFTGVVPILVELDGDVNGHKFSVSGEGEGDATYGKLTLKLICTTGKLPVPWPTLVTTLGYGLKCFARYPDHMKQHDFFKSAMPEGYVQERTIFFKDDGNYKTRAEVKFEGDTLVNRIELKGIGFKEDGNILGHKLEYNYYGKGLGIAVRKDNDALLQEINAALDKVKASPEYAQMQEKWFTQ

SEQ ID NO: 13 - protein, 473 aa, synthetic construct
ASVSARTLHFGTSATYAPYEFVDADNKIVGFDIDVANAVCKEMQAECSFTNQSFDSLIPSLRFKKFDAVIAGMDMTPKREQQVSFSQPYYEGLSAVVVTRKGAYHTFADLKGKKVGLENGTAHQRYLQDKQQAITPVAYDSYLNAFTDLKNNRLEGVFGDVAAIGKWLKNNPDYAIMDERASDYNSDNVYIMADKQKNGIKANFKIRHNVEDGSVQLADHYQQNTPIGDGPVLLPDNHYLSFQSVLSKDPNEKRDHMVLLEFVTAAGITLGMDELYNVDGGSGGTGSKGEELFTGVVPILVELDGDVNGHKFSVSGEGEGDATYGKLTLKLICTTGKLPVPWPTLVTTLGYGLKCFARYPDHMKQHDFFKSAMPEGYVQERTIFFKDDGNYKTRAEVKFEGDTLVNRIELKGIGFKEDGNILGHKLEYNYYGKGLGIAVRKDNDALLQEINAALDKVKASPEYAQMQEKWFTQ

SEQ ID NO: 14 - protein, 473 aa, synthetic construct
ASVSARTLHFGTSATYAPYEFVDADNKIVGFDIDVANAVCKEMQAECSFTNQSFDSLIPSLRFKKFDAVIAGMDMTPKREQQVSFSQPYYEGLSAVVVTRKGAYHTFADLKGKKVGLENGTTAQRYLQDKQQAITPVAYDSYLNAFTDLKNNRLEGVFGDVAAIGKWLKNNPDYAIMDERASDYNSDNVYIMADKQKNGIKANFKIRHNVEDGSVQLADHYQQNTPIGDGPVLLPDNHYLSFQSVLSKDPNEKRDHMVLLEFVTAAGITLGMDELYNVDGGSGGTGSKGEELFTGVVPILVELDGDVNGHKFSVSGEGEGDATYGKLTLKLICTTGKLPVPWPTLVTTLGYGLKCFARYPDHMKQHDFFKSAMPEGYVQERTIFFKDDGNYKTRAEVKFEGDTLVNRIELKGIGFKEDGNILGHKLEYNYYGKGLGIAVRKDNDALLQEINAALDKVKASPEYAQMQEKWFTQ

SEQ ID NO: 15 - protein, 473 aa, synthetic construct
ASVSARTLHFGTSATYAPYEFVDADNKIVGFDIDVANAVCKEMQAECSFTNQSFDSLIPSLRFKKFDAVIAGMDMTPKREQQVSFSQPYYEGLSAVVVTRKGAYHTFADLKGKKVGLENGTTHQRYLQDKQQAITPVAYDSYLNAFTDLKNNRLEGVFGAVAAIGKWLKNNPDYAIMDERASDYNSDNVYIMADKQKNGIKANFKIRHNVEDGSVQLADHYQQNTPIGDGPVLLPDNHYLSFQSVLSKDPNEKRDHMVLLEFVTAAGITLGMDELYNVDGGSGGTGSKGEELFTGVVPILVELDGDVNGHKFSVSGEGEGDATYGKLTLKLICTTGKLPVPWPTLVTTLGYGLKCFARYPDHMKQHDFFKSAMPEGYVQERTIFFKDDGNYKTRAEVKFEGDTLVNRIELKGIGFKEDGNILGHKLEYNYYGKGLGIAVRKDNDALLQEINAALDKVKASPEYAQMQEKWFTQ